European Patent Specification EP 3 911 751 B1, published February 26, 2025. Title: Liver-Specific Inducible Promoters and Methods of Use Thereof. Applicant: Synpromics Limited. The sequence listing filed with the application follows.

SEQUENCE LISTING (91 sequences)

SEQ ID NO: 1 - DNA, 51 bp, Mus musculus
tctgtactttcctgaccttggcacagtgccaccatcaacttgcctgacacc

SEQ ID NO: 2 - DNA, 51 bp, Homo sapiens
actgtactttcctgaccctgaagaggtggcagcatggactttcctgaacca

SEQ ID NO: 3 - DNA, 16 bp, Mus musculus
tgtactttcctgacct

SEQ ID NO: 4 - DNA, 16 bp, Homo sapiens
tgtactttcctgaccc

SEQ ID NO: 5 - DNA, 84 bp, Artificial Sequence
  3x NR1 sequence (mouse)
gatctctgtactttcctgaccttggatcgatctctgtactttcctgaccttggatcgatctctgtactttcctgaccttggatc

SEQ ID NO: 6 - DNA, 84 bp, Artificial Sequence
  3x NR1 sequence (human)
gatcactgtactttcctgaccctggatcgatcactgtactttcctgaccctggatcgatcactgtactttcctgaccctggatc

SEQ ID NO: 7 - DNA, 262 bp, Artificial Sequence
  PB1-MinTK
tctgtactttcctgaccttggcacagtgccaccatcaacttgcctgacaccgatccggccccgcccagcgtcttgtcattggcgaattcgaacacgcagatgcagtcggggcggcgcggtccgaggtccacttcgcatattaaggtgacgcgtgtggcctcgaacaccgagcgaccctgcagcgacccgcttaacagcgtcaacagcgtgccgcagatctcgaggagcttggcgagattttcaggagctaaggaagctaaac

SEQ ID NO: 8 - DNA, 180 bp, Artificial Sequence
  PB1-CMV-MP
tctgtactttcctgaccttggcacagtgccaccatcaacttgcctgacaccgctgggagttcgtagacggagcgattaatccatatgcaggtctatataagcagagctcgtttagtgaaccgtcagatcgcctagatacgccatccacgctgttttgacctccatagaagatcgccaccc

SEQ ID NO: 9 - DNA, 330 bp, Artificial Sequence
  PB1-SV40-MP
tctgtactttcctgaccttggcacagtgccaccatcaacttgcctgacaccgctgggagttcgtagacggactagcccgggctcgagatctgcgatctgcatctcaattagtcagcaaccatagtcccgcccctaactccgcccatcccgcccctaactccgcccagttccgcccattctccgccccatcgctgactaattttttttatttatgcagaggccgaggccgcctcggcctctgagctattccagaagtagtgaggaggcttttttggaggcctaggcttttgcaaaaagcttggcattccggtactgttggtaaagccaccc

SEQ ID NO: 10 - DNA, 353 bp, Artificial Sequence
  PB1-1-MinTk (2xPBREM)
tctgtactttcctgaccttggcacagtgccaccatcaacttgcctgacacccattactcgcatccattctctctgtactttcctgaccttggcacagtgccaccatcaacttgcctgacaccgctgggagttcgtagacggagatccggccccgcccagcgtcttgtcattggcgaattcgaacacgcagatgcagtcggggcggcgcggtccgaggtccacttcgcatattaaggtgacgcgtgtggcctcgaacaccgagcgaccctgcagcgacccgcttaacagcgtcaacagcgtgccgcagatctcgaggagcttggcgagattttcaggagctaaggaagctaaac

SEQ ID NO: 11 - DNA, 424 bp, Artificial Sequence
  PB1-2-MinTk (3xPBREM)
tctgtactttcctgaccttggcacagtgccaccatcaacttgcctgacacccattactcgcatccattctctctgtactttcctgaccttggcacagtgccaccatcaacttgcctgacaccgcactgaaggtcctcaatcgtctgtactttcctgaccttggcacagtgccaccatcaacttgcctgacaccgctgggagttcgtagacggagatccggccccgcccagcgtcttgtcattggcgaattcgaacacgcagatgcagtcggggcggcgcggtccgaggtccacttcgcatattaaggtgacgcgtgtggcctcgaacaccgagcgaccctgcagcgacccgcttaacagcgtcaacagcgtgccgcagatctcgaggagcttggcgagattttcaggagctaaggaagctaaac

SEQ ID NO: 12 - DNA, 495 bp, Artificial Sequence
  PB1-3-MinTk
tctgtactttcctgaccttggcacagtgccaccatcaacttgcctgacacccattactcgcatccattctctctgtactttcctgaccttggcacagtgccaccatcaacttgcctgacaccgcactgaaggtcctcaatcgtctgtactttcctgaccttggcacagtgccaccatcaacttgcctgacaccctgacctcctgccagcaatatctgtactttcctgaccttggcacagtgccaccatcaacttgcctgacaccgctgggagttcgtagacggagatccggccccgcccagcgtcttgtcattggcgaattcgaacacgcagatgcagtcggggcggcgcggtccgaggtccacttcgcatattaaggtgacgcgtgtggcctcgaacaccgagcgaccctgcagcgacccgcttaacagcgtcaacagcgtgccgcagatctcgaggagcttggcgagattttcaggagctaaggaagctaaac

SEQ ID NO: 13 - DNA, 401 bp, Artificial Sequence
  PB1-1-SV40
tctgtactttcctgaccttggcacagtgccaccatcaacttgcctgacacccattactcgcatccattctctctgtactttcctgaccttggcacagtgccaccatcaacttgcctgacaccgctgggagttcgtagacggactagcccgggctcgagatctgcgatctgcatctcaattagtcagcaaccatagtcccgcccctaactccgcccatcccgcccctaactccgcccagttccgcccattctccgccccatcgctgactaattttttttatttatgcagaggccgaggccgcctcggcctctgagctattccagaagtagtgaggaggcttttttggaggcctaggcttttgcaaaaagcttggcattccggtactgttggtaaagccaccc

SEQ ID NO: 14 - DNA, 472 bp, Artificial Sequence
  PB1-2-SV40
tctgtactttcctgaccttggcacagtgccaccatcaacttgcctgacacccattactcgcatccattctctctgtactttcctgaccttggcacagtgccaccatcaacttgcctgacaccgcactgaaggtcctcaatcgtctgtactttcctgaccttggcacagtgccaccatcaacttgcctgacaccgctgggagttcgtagacggactagcccgggctcgagatctgcgatctgcatctcaattagtcagcaaccatagtcccgcccctaactccgcccatcccgcccctaactccgcccagttccgcccattctccgccccatcgctgactaattttttttatttatgcagaggccgaggccgcctcggcctctgagctattccagaagtagtgaggaggcttttttggaggcctaggcttttgcaaaaagcttggcattccggtactgttggtaaagccaccc

SEQ ID NO: 15 - DNA, 543 bp, Artificial Sequence
  PB1-3-SV40
tctgtactttcctgaccttggcacagtgccaccatcaacttgcctgacacccattactcgcatccattctctctgtactttcctgaccttggcacagtgccaccatcaacttgcctgacaccgcactgaaggtcctcaatcgtctgtactttcctgaccttggcacagtgccaccatcaacttgcctgacaccctgacctcctgccagcaatatctgtactttcctgaccttggcacagtgccaccatcaacttgcctgacaccgctgggagttcgtagacggactagcccgggctcgagatctgcgatctgcatctcaattagtcagcaaccatagtcccgcccctaactccgcccatcccgcccctaactccgcccagttccgcccattctccgccccatcgctgactaattttttttatttatgcagaggccgaggccgcctcggcctctgagctattccagaagtagtgaggaggcttttttggaggcctaggcttttgcaaaaagcttggcattccggtactgttggtaaagccaccc

SEQ ID NO: 16 - DNA, 251 bp, Artificial Sequence
  PB1-1-CMV
tctgtactttcctgaccttggcacagtgccaccatcaacttgcctgacacccattactcgcatccattctctctgtactttcctgaccttggcacagtgccaccatcaacttgcctgacaccgctgggagttcgtagacggagcgattaatccatatgcaggtctatataagcagagctcgtttagtgaaccgtcagatcgcctagatacgccatccacgctgttttgacctccatagaagatcgccaccc

SEQ ID NO: 17 - DNA, 322 bp, Artificial Sequence
  PB1-2-CMV
tctgtactttcctgaccttggcacagtgccaccatcaacttgcctgacacccattactcgcatccattctctctgtactttcctgaccttggcacagtgccaccatcaacttgcctgacaccgcactgaaggtcctcaatcgtctgtactttcctgaccttggcacagtgccaccatcaacttgcctgacaccgctgggagttcgtagacggagcgattaatccatatgcaggtctatataagcagagctcgtttagtgaaccgtcagatcgcctagatacgccatccacgctgttttgacctccatagaagatcgccaccc

SEQ ID NO: 18 - DNA, 393 bp, Artificial Sequence
  PB1-3-CMV
tctgtactttcctgaccttggcacagtgccaccatcaacttgcctgacacccattactcgcatccattctctctgtactttcctgaccttggcacagtgccaccatcaacttgcctgacaccgcactgaaggtcctcaatcgtctgtactttcctgaccttggcacagtgccaccatcaacttgcctgacaccctgacctcctgccagcaatatctgtactttcctgaccttggcacagtgccaccatcaacttgcctgacaccgctgggagttcgtagacggagcgattaatccatatgcaggtctatataagcagagctcgtttagtgaaccgtcagatcgcctagatacgccatccacgctgttttgacctccatagaagatcgccaccc

SEQ ID NO: 19 - DNA, 1023 bp, Artificial Sequence
  PB1-MinTK and EPO
ggcctaactggccggtactctgtactttcctgaccttggcacagtgccaccatcaacttgcctgacaccgatccggccccgcccagcgtcttgtcattggcgaattcgaacacgcagatgcagtcggggcggcgcggtccgaggtccacttcgcatattaaggtgacgcgtgtggcctcgaacaccgagcgaccctgcagcgacccgcttaacagcgtcaacagcgtgccgcagatctcgaggagcttggcgagattttcaggagctaaggaagctaaacatgggggtgcacgaatgtcctgcctggctgtggcttctcctgtccctgctgtcgctccctctgggcctcccagtcctgggcgccccaccacgcctcatctgtgacagccgagtcctggagaggtacctcttggaggccaaggaggccgagaatatcacgacgggctgtgctgaacactgcagcttgaatgagaatatcactgtcccagacaccaaagttaatttctatgcctggaagaggatggaggtcgggcagcaggccgtagaagtctggcagggcctggccctgctgtcggaagctgtcctgcggggccaggccctgttggtcaactcttcccagccgtgggagcccctgcagctgcatgtggataaagccgtcagtggccttcgcagcctcaccactctgcttcgggctctgggagcccagaaggaagccatctcccctccagatgcggcctcagctgctccactccgaacaatcactgctgacactttccgcaaactcttccgagtctactccaatttcctccggggaaagctgaagctgtacacaggggaggcctgcaggacaggggacagatgatctagagtcggggcggccggccgcttcgagcagacatgataagatacattgatgagtttggacaaaccacaactagaatgcagtgaaaaaaatgctttatttgtgaaatttgtgatgctattgctttatttgtaaccattataagctgcaataaacaagtt

SEQ ID NO: 20 - DNA, 16 bp, Artificial Sequence
  NR1 motif from PBREM
  misc_feature (16)..(16): n is a, c, g, or t
tgtactttcctgaccn

SEQ ID NO: 21 - DNA, 17 bp, Artificial Sequence
  sequence preferably comprised in a functional variant of a PBREM element
  misc_feature (17)..(17): n is a, c, g, or t
ctgtactttcctgaccn

SEQ ID NO: 22 - DNA, 17 bp, Artificial Sequence
  sequence preferably comprised in a functional variant of a PBREM element
ctgtactttcctgaccy

SEQ ID NO: 23 - DNA, 17 bp, Artificial Sequence
  sequence preferably comprised in a functional variant of a PBREM element
ctgtactttcctgacct

SEQ ID NO: 24 - DNA, 17 bp, Artificial Sequence
  sequence preferably comprised in a functional variant of a PBREM element
ctgtactttcctgaccc

SEQ ID NO: 25 - DNA, 20 bp, Artificial Sequence
  sequence suitably comprised in a functional variant of a PBREM sequence
  misc_feature (1)..(1): n is a, c, g, or t
  misc_feature (18)..(18): n is a, c, g, or t
nctgtactttcctgaccntg

SEQ ID NO: 26 - DNA, 20 bp, Artificial Sequence
  sequence suitably comprised in a functional variant of a PBREM sequence
wctgtactttcctgaccytg

SEQ ID NO: 27 - DNA, 20 bp, Artificial Sequence
  sequence suitably comprised in a functional variant of a PBREM sequence
tctgtactttcctgaccttg

SEQ ID NO: 28 - DNA, 20 bp, Artificial Sequence
  sequence suitably comprised in a functional variant of a PBREM sequence
actgtactttcctgaccctg

SEQ ID NO: 29 - DNA, 16 bp, Artificial Sequence
  sequence suitably comprised in a functional variant of a PBREM sequence
  misc_feature (16)..(16): optional spacer
  misc_feature (16)..(16): n is a, c, g, or t
tgtactttcctgaccn

SEQ ID NO: 30 - DNA, 17 bp, Artificial Sequence
  sequence suitably comprised in a functional variant of a PBREM sequence
  misc_feature (17)..(17): optional spacer
  misc_feature (17)..(17): n is a, c, g, or t
ctgtactttcctgaccn

SEQ ID NO: 31 - DNA, 20 bp, Artificial Sequence
  sequence suitably comprised in a functional variant of a PBREM sequence
  misc_feature (1)..(1): n is a, c, g, or t
  misc_feature (18)..(18): n is a, c, g, or t
  misc_feature (20)..(20): optional spacer
nctgtactttcctgaccntg

SEQ ID NO: 32 - DNA, 32 bp, Artificial Sequence
  sequence suitably comprised in a functional variant of a PBREM sequence
  misc_feature (16)..(17): optional spacer
  misc_feature (16)..(16): n is a, c, g, or t
  misc_feature (32)..(32): n is a, c, g, or t
tgtactttcctgaccntgtactttcctgaccn

SEQ ID NO: 33 - DNA, 48 bp, Artificial Sequence
  sequence suitably comprised in a functional variant of a PBREM sequence
  misc_feature (16)..(17): optional spacer
  misc_feature (16)..(16): n is a, c, g, or t
  misc_feature (32)..(32): n is a, c, g, or t
  misc_feature (32)..(33): optional spacer
  misc_feature (48)..(48): n is a, c, g, or t
tgtactttcctgaccntgtactttcctgaccntgtactttcctgaccn

SEQ ID NO: 34 - DNA, 34 bp, Artificial Sequence
  sequence suitably comprised in a functional variant of a PBREM sequence
  misc_feature (17)..(18): optional spacer
  misc_feature (17)..(17): n is a, c, g, or t
  misc_feature (34)..(34): n is a, c, g, or t
ctgtactttcctgaccnctgtactttcctgaccn

SEQ ID NO: 35 - DNA, 51 bp, Artificial Sequence
  sequence suitably comprised in a functional variant of a PBREM sequence
  misc_feature (17)..(18): optional spacer
  misc_feature (17)..(17): n is a, c, g, or t
  misc_feature (34)..(34): n is a, c, g, or t
  misc_feature (34)..(35): optional spacer
  misc_feature (51)..(51): n is a, c, g, or t
ctgtactttcctgaccnctgtactttcctgaccnctgtactttcctgaccn

SEQ ID NO: 36 - DNA, 40 bp, Artificial Sequence
  sequence suitably comprised in a functional variant of a PBREM sequence
  misc_feature (1)..(1): n is a, c, g, or t
  misc_feature (18)..(18): n is a, c, g, or t
  misc_feature (20)..(21): optional spacer
  misc_feature (21)..(21): n is a, c, g, or t
  misc_feature (38)..(38): n is a, c, g, or t
nctgtactttcctgaccntgnctgtactttcctgaccntg

SEQ ID NO: 37 - DNA, 60 bp, Artificial Sequence
  sequence suitably comprised in a functional variant of a PBREM sequence
  misc_feature (1)..(1): n is a, c, g, or t
  misc_feature (18)..(18): n is a, c, g, or t
  misc_feature (20)..(21): optional spacer
  misc_feature (21)..(21): n is a, c, g, or t
  misc_feature (38)..(38): n is a, c, g, or t
  misc_feature (40)..(41): optional spacer
  misc_feature (41)..(41): n is a, c, g, or t
  misc_feature (58)..(58): n is a, c, g, or t
nctgtactttcctgaccntgnctgtactttcctgaccntgnctgtactttcctgaccntg

SEQ ID NO: 38 - DNA, 60 bp, Artificial Sequence
  sequence suitably comprised in a functional variant of a PBREM sequence
  misc_feature (20)..(21): optional spacer
  misc_feature (40)..(41): optional spacer
tctgtactttcctgaccttgtctgtactttcctgaccttgtctgtactttcctgaccttg

SEQ ID NO: 39 - DNA, 60 bp, Artificial Sequence
  sequence suitably comprised in a functional variant of a PBREM sequence
  misc_feature (20)..(21): optional spacer
  misc_feature (40)..(41): optional spacer
actgtactttcctgaccctgactgtactttcctgaccctgactgtactttcctgaccctg

SEQ ID NO: 40 - DNA, 8 bp, Artificial Sequence
  spacer
gatcgatc

SEQ ID NO: 41 - DNA, 51 bp, Artificial Sequence
  sequence preferably comprised in a functional variant of a PBREM sequence
  misc_feature (1)..(1): n is a, c, g, or t
  misc_feature (18)..(18): n is a, c, g, or t
  misc_feature (21)..(25): n is a, c, g, or t
  misc_feature (29)..(29): n is a, c, g, or t
  misc_feature (32)..(32): n is a, c, g, or t
  misc_feature (36)..(37): n is a, c, g, or t
  misc_feature (42)..(42): n is a, c, g, or t
  misc_feature (48)..(49): n is a, c, g, or t
  misc_feature (51)..(51): n is a, c, g, or t
nctgtactttcctgaccntgnnnnngtgncancatnnacttncctganncn

SEQ ID NO: 42 - DNA, 102 bp, Artificial Sequence
  CRM
  misc_feature (1)..(1): n is a, c, g, or t
  misc_feature (18)..(18): n is a, c, g, or t
  misc_feature (21)..(25): n is a, c, g, or t
  misc_feature (29)..(29): n is a, c, g, or t
  misc_feature (32)..(32): n is a, c, g, or t
  misc_feature (36)..(37): n is a, c, g, or t
  misc_feature (42)..(42): n is a, c, g, or t
  misc_feature (48)..(49): n is a, c, g, or t
  misc_feature (51)..(52): optional spacer
  misc_feature (51)..(51): n is a, c, g, or t
  misc_feature (52)..(52): n is a, c, g, or t
  misc_feature (69)..(69): n is a, c, g, or t
  misc_feature (72)..(76): n is a, c, g, or t
  misc_feature (80)..(80): n is a, c, g, or t
  misc_feature (83)..(83): n is a, c, g, or t
  misc_feature (87)..(88): n is a, c, g, or t
  misc_feature (93)..(93): n is a, c, g, or t
  misc_feature (99)..(100): n is a, c, g, or t
  misc_feature (102)..(102): n is a, c, g, or t
nctgtactttcctgaccntgnnnnngtgncancatnnacttncctganncnnctgtactttcctgaccntgnnnnngtgncancatnnacttncctganncn

SEQ ID NO: 43 - DNA, 153 bp, Artificial Sequence
  CRM
  misc_feature (1)..(1): n is a, c, g, or t
  misc_feature (18)..(18): n is a, c, g, or t
  misc_feature (21)..(25): n is a, c, g, or t
  misc_feature (29)..(29): n is a, c, g, or t
  misc_feature (32)..(32): n is a, c, g, or t
  misc_feature (36)..(37): n is a, c, g, or t
  misc_feature (42)..(42): n is a, c, g, or t
  misc_feature (48)..(49): n is a, c, g, or t
  misc_feature (51)..(52): optional spacer
  misc_feature (51)..(51): n is a, c, g, or t
  misc_feature (52)..(52): n is a, c, g, or t
  misc_feature (69)..(69): n is a, c, g, or t
  misc_feature (72)..(76): n is a, c, g, or t
  misc_feature (80)..(80): n is a, c, g, or t
  misc_feature (83)..(83): n is a, c, g, or t
  misc_feature (87)..(88): n is a, c, g, or t
  misc_feature (93)..(93): n is a, c, g, or t
  misc_feature (99)..(100): n is a, c, g, or t
  misc_feature (102)..(102): n is a, c, g, or t
  misc_feature (102)..(103): optional spacer
  misc_feature (103)..(103): n is a, c, g, or t
  misc_feature (120)..(120): n is a, c, g, or t
  misc_feature (123)..(127): n is a, c, g, or t
  misc_feature (131)..(131): n is a, c, g, or t
  misc_feature (134)..(134): n is a, c, g, or t
  misc_feature (138)..(139): n is a, c, g, or t
  misc_feature (144)..(144): n is a, c, g, or t
  misc_feature (150)..(151): n is a, c, g, or t
  misc_feature (153)..(153): n is a, c, g, or t
nctgtactttcctgaccntgnnnnngtgncancatnnacttncctganncnnctgtactttcctgaccntgnnnnngtgncancatnnacttncctganncnnctgtactttcctgaccntgnnnnngtgncancatnnacttncctganncn

SEQ ID NO: 44 - DNA, 102 bp, Artificial Sequence
  CRM
  misc_feature (51)..(52): optional spacer
tctgtactttcctgaccttggcacagtgccaccatcaacttgcctgacacctctgtactttcctgaccttggcacagtgccaccatcaacttgcctgacacc

SEQ ID NO: 45 - DNA, 153 bp, Artificial Sequence
  CRM
  misc_feature (51)..(52): optional spacer
  misc_feature (102)..(103): optional spacer
tctgtactttcctgaccttggcacagtgccaccatcaacttgcctgacacctctgtactttcctgaccttggcacagtgccaccatcaacttgcctgacacctctgtactttcctgaccttggcacagtgccaccatcaacttgcctgacacc

SEQ ID NO: 46 - DNA, 153 bp, Artificial Sequence
  CRM
  misc_feature (51)..(52): optional spacer
  misc_feature (102)..(103): optional spacer
actgtactttcctgaccctgaagaggtggcagcatggactttcctgaaccaactgtactttcctgaccctgaagaggtggcagcatggactttcctgaaccaactgtactttcctgaccctgaagaggtggcagcatggactttcctgaacca

SEQ ID NO: 47 - DNA, 102 bp, Artificial Sequence
  CRM
  misc_feature (51)..(52): optional spacer
actgtactttcctgaccctgaagaggtggcagcatggactttcctgaaccaactgtactttcctgaccctgaagaggtggcagcatggactttcctgaacca

SEQ ID NO: 48 - DNA, 5716 bp, Artificial Sequence
  pAAV-ZsGreen original plasmid
agcgcccaatacgcaaaccgcctctccccgcgcgttggccgattcattaatgcagctggcacgacaggtttcccgactggaaagcgggcagtgagcgcaacgcaattaatgtgagttagctcactcattaggcaccccaggctttacactttatgcttccggctcgtatgttgtgtggaattgtgagcggataacaatttcacacaggaaacagctatgaccatgattacgaattgcctgcaggcagctgcgcgctcgctcgctcactgaggccgcccgggcaaagcccgggcgtcgggcgacctttggtcgcccggcctcagtgagcgagcgagcgcgcagagagggagtggccaactccatcactaggggttcctatcgatatcaagctttaatagtaatcaattacggggtcattagttcatagcccatatatggagttccgcgttacataacttacggtaaatggcccgcctggctgaccgcccaacgacccccgcccattgacgtcaataatgacgtatgttcccatagtaacgccaatagggactttccattgacgtcaatgggtggagtatttacggtaaactgcccacttggcagtacatcaagtgtatcatatgccaagtacgccccctattgacgtcaatgacggtaaatggcccgcctggcattatgcccagtacatgaccttatgggactttcctacttggcagtacatctacgtattagtcatcgctattaccatggtgatgcggttttggcagtacatcaatgggcgtggatagcggtttgactcacggggatttccaagtctccaccccattgacgtcaatgggagtttgttttggcaccaaaatcaacgggactttccaaaatgtcgtaacaactccgccccattgacgcaaatgggcggtaggcgtgtacggtgggaggtctatataagcagagctggtttagtggatatccttaagggcccagccggcccgaatcccggccgggaacggtgcattggaacgcggattccccgtgccaagagtgacgtaagtaccgcctatagagtctataggcccacaaaaaatgctttcttcttttaatatacttttttgtttatcttatttctaatactttccctaatctctttctttcagggcaataatgatacaatgtatcatgcctctttgcaccattctaaagaataacagtgataatttctgggttaaggcaatagcaatatttctgcatataaatatttctgcatataaattgtaactgatgtaagaggtttcatattgctaatagcagctacaatccagctaccattctgcttttattttatggttgggataaggctggattattctgagtccaagctaggcccttttgctaatcatgttcatacctcttatcttcctcccacagctcctgggcaacgtgctggtctgtgtgctggcccatcactttggcaaagaattgggattcgcgagaattcgccaccatggcccagtccaagcacggcctgaccaaggagatgaccatgaagtaccgcatggagggctgcgtggacggccacaagttcgtgatcaccggcgagggcatcggctaccccttcaagggcaagcaggccatcaacctgtgcgtggtggagggcggccccttgcccttcgccgaggacatcttgtccgccgccttcatgtacggcaaccgcgtgttcaccgagtacccccaggacatcgtcgactacttcaagaactcctgccccgccggctacacctgggaccgctccttcctgttcgaggacggcgccgtgtgcatctgcaacgccgacatcaccgtgagcgtggaggagaactgcatgtaccacgagtccaagttctacggcgtgaacttccccgccgacggccccgtgatgaagaagatgaccgacaactgggagccctcctgcgagaagatcatccccgtgcccaagcagggcatcttgaagggcgacgtgagcatgtacctgctgctgaaggacggtggccgcttgcgctgccagttcgacaccgtgtacaaggccaagtccgtgccccgcaagatgcccgactggcacttcatccagcacaagctgacccgcgaggaccgcagcgacgccaagaaccagaagtggcacctgaccgagcacgccatcgcctccggctccgccttgccctgataaggatccacgggtggcatccctgtgacccctccccagtgcctctcctggccctggaagttgccactccagtgcccaccagccttgtcctaataaaattaagttgcatcattttgtctgactaggtgtccttctataatattatggggtggaggggggtggtatggagcaaggggcaagttgggaagacaacctgtagggcctgcggggtctattgggaaccaagctggagtgcagtggcacaatcttggctcactgcaatctccgcctcctgggttcaagcgattctcctgcctcagcctcccgagttgttgggattccaggcatgcatgaccaggctcagctaatttttgtttttttggtagagacggggtttcaccatattggccaggctggtctccaactcctaatctcaggtgatctacccaccttggcctcccaaattgctgggattacaggcgtgaaccactgctcccttccctgtccttatcgatagatctaggaacccctagtgatggagttggccactccctctctgcgcgctcgctcgctcactgaggccgggcgaccaaaggtcgcccgacgcccgggctttgcccgggcggcctcagtgagcgagcgagcgcgcagctgcctgcaggcagcttggcactggccgtcgttttacaacgtcgtgactgggaaaaccctggcgttacccaacttaatcgccttgcagcacatccccctttcgccagctggcgtaatagcgaagaggcccgcaccgatcgcccttcccaacagttgcgcagcctgaatggcgaatggcgcctgatgcggtattttctccttacgcatctgtgcggtatttcacaccgcatacgtcaaagcaaccatagtacgcgccctgtagcggcgcattaagcgcggcgggtgtggtggttacgcgcagcgtgaccgctacacttgccagcgccctagcgcccgctcctttcgctttcttcccttcctttctcgccacgttcgccggctttccccgtcaagctctaaatcgggggctccctttagggttccgatttagtgctttacggcacctcgaccccaaaaaacttgatttgggtgatggttcacgtagtgggccatcgccctgatagacggtttttcgccctttgacgttggagtccacgttctttaatagtggactcttgttccaaactggaacaacactcaaccctatctcgggctattcttttgatttataagggattttgccgatttcggcctattggttaaaaaatgagctgatttaacaaaaatttaacgcgaattttaacaaaatattaacgtttacaattttatggtgcactctcagtacaatctgctctgatgccgcatagttaagccagccccgacacccgccaacacccgctgacgcgccctgacgggcttgtctgctcccggcatccgcttacagacaagctgtgaccgtctccgggagctgcatgtgtcagaggttttcaccgtcatcaccgaaacgcgcgagacgaaagggcctcgtgatacgcctatttttataggttaatgtcatgataataatggtttcttagacgtcaggtggcacttttcggggaaatgtgcgcggaacccctatttgtttatttttctaaatacattcaaatatgtatccgctcatgagacaataaccctgataaatgcttcaataatattgaaaaaggaagagtatgagtattcaacatttccgtgtcgcccttattcccttttttgcggcattttgccttcctgtttttgctcacccagaaacgctggtgaaagtaaaagatgctgaagatcagttgggtgcacgagtgggttacatcgaactggatctcaacagcggtaagatccttgagagttttcgccccgaagaacgttttccaatgatgagcacttttaaagttctgctatgtggcgcggtattatcccgtattgacgccgggcaagagcaactcggtcgccgcatacactattctcagaatgacttggttgagtactcaccagtcacagaaaagcatcttacggatggcatgacagtaagagaattatgcagtgctgccataaccatgagtgataacactgcggccaacttacttctgacaacgatcggaggaccgaaggagctaaccgcttttttgcacaacatgggggatcatgtaactcgccttgatcgttgggaaccggagctgaatgaagccataccaaacgacgagcgtgacaccacgatgcctgtagcaatggcaacaacgttgcgcaaactattaactggcgaactacttactctagcttcccggcaacaattaatagactggatggaggcggataaagttgcaggaccacttctgcgctcggcccttccggctggctggtttattgctgataaatctggagccggtgagcgtgggtctcgcggtatcattgcagcactggggccagatggtaagccctcccgtatcgtagttatctacacgacggggagtcaggcaactatggatgaacgaaatagacagatcgctgagataggtgcctcactgattaagcattggtaactgtcagaccaagtttactcatatatactttagattgatttaaaacttcatttttaatttaaaaggatctaggtgaagatcctttttgataatctcatgaccaaaatcccttaacgtgagttttcgttccactgagcgtcagaccccgtagaaaagatcaaaggatcttcttgagatcctttttttctgcgcgtaatctgctgcttgcaaacaaaaaaaccaccgctaccagcggtggtttgtttgccggatcaagagctaccaactctttttccgaaggtaactggcttcagcagagcgcagataccaaatactgttcttctagtgtagccgtagttaggccaccacttcaagaactctgtagcaccgcctacatacctcgctctgctaatcctgttaccagtggctgctgccagtggcgataagtcgtgtcttaccgggttggactcaagacgatagttaccggataaggcgcagcggtcgggctgaacggggggttcgtgcacacagcccagcttggagcgaacgacctacaccgaactgagatacctacagcgtgagctatgagaaagcgccacgcttcccgaagggagaaaggcggacaggtatccggtaagcggcagggtcggaacaggagagcgcacgagggagcttccagggggaaacgcctggtatctttatagtcctgtcgggtttcgccacctctgacttgagcgtcgatttttgtgatgctcgtcaggggggcggagcctatggaaaaacgccagcaacgcggcctttttacggttcctggccttttgctggccttttgctcacatgttctttcctgcgttatcccctgattctgtggataaccgtattaccgcctttgagtgagctgataccgctcgccgcagccgaacgaccgagcgcagcgagtcagtgagcgaggaagcggaag

SEQ ID NO: 49 - DNA, 5857 bp, Artificial Sequence
  pAAV-PB1-MinTk
tgcctgcaggcagctgcgcgctcgctcgctcactgaggccgcccgggcaaagcccgggcgtcgggcgacctttggtcgcccggcctcagtgagcgagcgagcgcgcagagagggagtggccaactccatcactaggggttcctatcgatatcaagcttctgtactttcctgaccttggcacagtgccaccatcaacttgcctgacaccgatccggccccgcccagcgtcttgtcattggcgaattcgaacacgcagatgcagtcggggcggcgcggtccgaggtccacttcgcatattaaggtgacgcgtgtggcctcgaacaccgagcgaccctgcagcgacccgcttaacagcgtcaacagcgtgccgcagatctcgaggagcttggcgagattttcaggagctaaggaagctaaacatggaagatgccaaaaacattaagaagggcccagcgccattctacccactcgaagacgggaccgccggcgagcagctgcacaaagccatgaagcgctacgccctggtgcccggcaccatcgcctttaccgacgcacatatcgaggtggacattacctacgccgagtacttcgagatgagcgttcggctggcagaagctatgaagcgctatgggctgaatacaaaccatcggatcgtggtgtgcagcgagaatagcttgcagttcttcatgcccgtgttgggtgccctgttcatcggtgtggctgtggccccagctaacgacatctacaacgagcgcgagctgctgaacagcatgggcatcagccagcccaccgtcgtattcgtgagcaagaaagggctgcaaaagatcctcaacgtgcaaaagaagctaccgatcatacaaaagatcatcatcatggatagcaagaccgactaccagggcttccaaagcatgtacaccttcgtgacttcccatttgccacccggcttcaacgagtacgacttcgtgcccgagagcttcgaccgggacaaaaccatcgccctgatcatgaacagtagtggcagtaccggattgcccaagggcgtagccctaccgcaccgcaccgcttgtgtccgattcagtcatgcccgcgaccccatcttcggcaaccagatcatccccgacaccgctatcctcagcgtggtgccatttcaccacggcttcggcatgttcaccacgctgggctacttgatctgcggctttcgggtcgtgctcatgtaccgcttcgaggaggagctattcttgcgcagcttgcaagactataagattcaatctgccctgctggtgcccacactatttagcttcttcgctaagagcactctcatcgacaagtacgacctaagcaacttgcacgagatcgccagcggcggggcgccgctcagcaaggaggtaggtgaggccgtggccaaacgcttccacctaccaggcatccgccagggctacggcctgacagaaacaaccagcgccattctgatcacccccgaaggggacgacaagcctggcgcagtaggcaaggtggtgcccttcttcgaggctaaggtggtggacttggacaccggtaagacactgggtgtgaaccagcgcggcgagctgtgcgtccgtggccccatgatcatgagcggctacgttaacaaccccgaggctacaaacgctctcatcgacaaggacggctggctgcacagcggcgacatcgcctactgggacgaggacgagcacttcttcatcgtggaccggctgaagagcctgatcaaatacaagggctaccaggtagccccagccgaactggagagcatcctgctgcaacaccccaacatcttcgacgccggggtcgccggcctgcccgacgacgatgccggcgagctgcccgccgcagtcgtcgtgctggaacacggtaaaaccatgaccgagaaggagatcgtggactatgtggccagccaggttacaaccgccaagaagctgcgcggtggtgttgtgttcgtggacgaggtgcctaaaggactgaccggcaagttggacgcccgcaagatccgcgagattctcattaaggccaagaagggcggcaagatcgccgtgtaatcgcgagaattctctagagtcgacactagtgcggatccacgggtggcatccctgtgacccctccccagtgcctctcctggccctggaagttgccactccagtgcccaccagccttgtcctaataaaattaagttgcatcattttgtctgactaggtgtccttctataatattatggggtggaggggggtggtatggagcaaggggcaagttgggaagacaacctgtagggcctgcggggtctattgggaaccaagctggagtgcagtggcacaatcttggctcactgcaatctccgcctcctgggttcaagcgattctcctgcctcagcctcccgagttgttgggattccaggcatgcatgaccaggctcagctaatttttgtttttttggtagagacggggtttcaccatattggccaggctggtctccaactcctaatctcaggtgatctacccaccttggcctcccaaattgctgggattacaggcgtgaaccactgctcccttccctgtccttatcgatagatctaggaacccctagtgatggagttggccactccctctctgcgcgctcgctcgctcactgaggccgggcgaccaaaggtcgcccgacgcccgggctttgcccgggcggcctcagtgagcgagcgagcgcgcagctgcctgcaggcagcttggcactggccgtcgttttacaacgtcgtgactgggaaaaccctggcgttacccaacttaatcgccttgcagcacatccccctttcgccagctggcgtaatagcgaagaggcccgcaccgatcgcccttcccaacagttgcgcagcctgaatggcgaatggcgcctgatgcggtattttctccttacgcatctgtgcggtatttcacaccgcatacgtcaaagcaaccatagtacgcgccctgtagcggcgcattaagcgcggcgggtgtggtggttacgcgcagcgtgaccgctacacttgccagcgccctagcgcccgctcctttcgctttcttcccttcctttctcgccacgttcgccggctttccccgtcaagctctaaatcgggggctccctttagggttccgatttagtgctttacggcacctcgaccccaaaaaacttgatttgggtgatggttcacgtagtgggccatcgccctgatagacggtttttcgccctttgacgttggagtccacgttctttaatagtggactcttgttccaaactggaacaacactcaaccctatctcgggctattcttttgatttataagggattttgccgatttcggcctattggttaaaaaatgagctgatttaacaaaaatttaacgcgaattttaacaaaatattaacgtttacaattttatggtgcactctcagtacaatctgctctgatgccgcatagttaagccagccccgacacccgccaacacccgctgacgcgccctgacgggcttgtctgctcccggcatccgcttacagacaagctgtgaccgtctccgggagctgcatgtgtcagaggttttcaccgtcatcaccgaaacgcgcgagacgaaagggcctcgtgatacgcctatttttataggttaatgtcatgataataatggtttcttagacgtcaggtggcacttttcggggaaatgtgcgcggaacccctatttgtttatttttctaaatacattcaaatatgtatccgctcatgagacaataaccctgataaatgcttcaataatattgaaaaaggaagagtatgagtattcaacatttccgtgtcgcccttattcccttttttgcggcattttgccttcctgtttttgctcacccagaaacgctggtgaaagtaaaagatgctgaagatcagttgggtgcacgagtgggttacatcgaactggatctcaacagcggtaagatccttgagagttttcgccccgaagaacgttttccaatgatgagcacttttaaagttctgctatgtggcgcggtattatcccgtattgacgccgggcaagagcaactcggtcgccgcatacactattctcagaatgacttggttgagtactcaccagtcacagaaaagcatcttacggatggcatgacagtaagagaattatgcagtgctgccataaccatgagtgataacactgcggccaacttacttctgacaacgatcggaggaccgaaggagctaaccgcttttttgcacaacatgggggatcatgtaactcgccttgatcgttgggaaccggagctgaatgaagccataccaaacgacgagcgtgacaccacgatgcctgtagcaatggcaacaacgttgcgcaaactattaactggcgaactacttactctagcttcccggcaacaattaatagactggatggaggcggataaagttgcaggaccacttctgcgctcggcccttccggctggctggtttattgctgataaatctggagccggtgagcgtgggtctcgcggtatcattgcagcactggggccagatggtaagccctcccgtatcgtagttatctacacgacggggagtcaggcaactatggatgaacgaaatagacagatcgctgagataggtgcctcactgattaagcattggtaactgtcagaccaagtttactcatatatactttagattgatttaaaacttcatttttaatttaaaaggatctaggtgaagatcctttttgataatctcatgaccaaaatcccttaacgtgagttttcgttccactgagcgtcagaccccgtagaaaagatcaaaggatcttcttgagatcctttttttctgcgcgtaatctgctgcttgcaaacaaaaaaaccaccgctaccagcggtggtttgtttgccggatcaagagctaccaactctttttccgaaggtaactggcttcagcagagcgcagataccaaatactgttcttctagtgtagccgtagttaggccaccacttcaagaactctgtagcaccgcctacatacctcgctctgctaatcctgttaccagtggctgctgccagtggcgataagtcgtgtcttaccgggttggactcaagacgatagttaccggataaggcgcagcggtcgggctgaacggggggttcgtgcacacagcccagcttggagcgaacgacctacaccgaactgagatacctacagcgtgagctatgagaaagcgccacgcttcccgaagggagaaaggcggacaggtatccggtaagcggcagggtcggaacaggagagcgcacgagggagcttccagggggaaacgcctggtatctttatagtcctgtcgggtttcgccacctctgacttgagcgtcgatttttgtgatgctcgtcaggggggcggagcctatggaaaaacgccagcaacgcggcctttttacggttcctggccttttgctggccttttgctcacatgttctttcctgcgttatcccctgattctgtggataaccgtattaccgcctttgagtgagctgataccgctcgccgcagccgaacgaccgagcgcagcgagtcagtgagcgaggaagcggaagagcgcccaatacgcaaaccgcctctccccgcgcgttggccgattcattaatgcagctggcacgacaggtttcccgactggaaagcgggcagtgagcgcaacgcaattaatgtgagttagctcactcattaggcaccccaggctttacactttatgcttccggctcgtatgttgtgtggaattgtgagcggataacaatttcacacaggaaacagctatgaccatgattacgaat

SEQ ID NO: 50 - DNA, 6044 bp, Artificial Sequence
  pAAV-PB1-2-MinTk
gcctgcaggcagctgcgcgctcgctcgctcactgaggccgcccgggcaaagcccgggcgtcgggcgacctttggtcgcccggcctcagtgagcgagcgagcgcgcagagagggagtggccaactccatcactaggggttcctatcgatatcaagcttttctctggcctaactggccggtactctgtactttcctgaccttggcacagtgccaccatcaacttgcctgacacccattactcgcatccattctctctgtactttcctgaccttggcacagtgccaccatcaacttgcctgacaccgcactgaaggtcctcaatcgtctgtactttcctgaccttggcacagtgccaccatcaacttgcctgacaccgctgggagttcgtagacggagatccggccccgcccagcgtcttgtcattggcgaattcgaacacgcagatgcagtcggggcggcgcggtccgaggtccacttcgcatattaaggtgacgcgtgtggcctcgaacaccgagcgaccctgcagcgacccgcttaacagcgtcaacagcgtgccgcagatctcgaggagcttggcgagattttcaggagctaaggaagctaaacatggaagatgccaaaaacattaagaagggcccagcgccattctacccactcgaagacgggaccgccggcgagcagctgcacaaagccatgaagcgctacgccctggtgcccggcaccatcgcctttaccgacgcacatatcgaggtggacattacctacgccgagtacttcgagatgagcgttcggctggcagaagctatgaagcgctatgggctgaatacaaaccatcggatcgtggtgtgcagcgagaatagcttgcagttcttcatgcccgtgttgggtgccctgttcatcggtgtggctgtggccccagctaacgacatctacaacgagcgcgagctgctgaacagcatgggcatcagccagcccaccgtcgtattcgtgagcaagaaagggctgcaaaagatcctcaacgtgcaaaagaagctaccgatcatacaaaagatcatcatcatggatagcaagaccgactaccagggcttccaaagcatgtacaccttcgtgacttcccatttgccacccggcttcaacgagtacgacttcgtgcccgagagcttcgaccgggacaaaaccatcgccctgatcatgaacagtagtggcagtaccggattgcccaagggcgtagccctaccgcaccgcaccgcttgtgtccgattcagtcatgcccgcgaccccatcttcggcaaccagatcatccccgacaccgctatcctcagcgtggtgccatttcaccacggcttcggcatgttcaccacgctgggctacttgatctgcggctttcgggtcgtgctcatgtaccgcttcgaggaggagctattcttgcgcagcttgcaagactataagattcaatctgccctgctggtgcccacactatttagcttcttcgctaagagcactctcatcgacaagtacgacctaagcaacttgcacgagatcgccagcggcggggcgccgctcagcaaggaggtaggtgaggccgtggccaaacgcttccacctaccaggcatccgccagggctacggcctgacagaaacaaccagcgccattctgatcacccccgaaggggacgacaagcctggcgcagtaggcaaggtggtgcccttcttcgaggctaaggtggtggacttggacaccggtaagacactgggtgtgaaccagcgcggcgagctgtgcgtccgtggccccatgatcatgagcggctacgttaacaaccccgaggctacaaacgctctcatcgacaaggacggctggctgcacagcggcgacatcgcctactgggacgaggacgagcacttcttcatcgtggaccggctgaagagcctgatcaaatacaagggctaccaggtagccccagccgaactggagagcatcctgctgcaacaccccaacatcttcgacgccggggtcgccggcctgcccgacgacgatgccggcgagctgcccgccgcagtcgtcgtgctggaacacggtaaaaccatgaccgagaaggagatcgtggactatgtggccagccaggttacaaccgccaagaagctgcgcggtggtgttgtgttcgtggacgaggtgcctaaaggactgaccggcaagttggacgcccgcaagatccgcgagattctcattaaggccaagaagggcggcaagatcgccgtgtaatcgcgagaattctctagagtcgacactagtgcggatccacgggtggcatccctgtgacccctccccagtgcctctcctggccctggaagttgccactccagtgcccaccagccttgtcctaataaaattaagttgcatcattttgtctgactaggtgtccttctataatattatggggtggaggggggtggtatggagcaaggggcaagttgggaagacaacctgtagggcctgcggggtctattgggaaccaagctggagtgcagtggcacaatcttggctcactgcaatctccgcctcctgggttcaagcgattctcctgcctcagcctcccgagttgttgggattccaggcatgcatgaccaggctcagctaatttttgtttttttggtagagacggggtttcaccatattggccaggctggtctccaactcctaatctcaggtgatctacccaccttggcctcccaaattgctgggattacaggcgtgaaccactgctcccttccctgtccttatcgatagatctaggaacccctagtgatggagttggccactccctctctgcgcgctcgctcgctcactgaggccgggcgaccaaaggtcgcccgacgcccgggctttgcccgggcggcctcagtgagcgagcgagcgcgcagctgcctgcaggcagcttggcactggccgtcgttttacaacgtcgtgactgggaaaaccctggcgttacccaacttaatcgccttgcagcacatccccctttcgccagctggcgtaatagcgaagaggcccgcaccgatcgcccttcccaacagttgcgcagcctgaatggcgaatggcgcctgatgcggtattttctccttacgcatctgtgcggtatttcacaccgcatacgtcaaagcaaccatagtacgcgccctgtagcggcgcattaagcgcggcgggtgtggtggttacgcgcagcgtgaccgctacacttgccagcgccctagcgcccgctcctttcgctttcttcccttcctttctcgccacgttcgccggctttccccgtcaagctctaaatcgggggctccctttagggttccgatttagtgctttacggcacctcgaccccaaaaaacttgatttgggtgatggttcacgtagtgggccatcgccctgatagacggtttttcgccctttgacgttggagtccacgttctttaatagtggactcttgttccaaactggaacaacactcaaccctatctcgggctattcttttgatttataagggattttgccgatttcggcctattggttaaaaaatgagctgatttaacaaaaatttaacgcgaattttaacaaaatattaacgtttacaattttatggtgcactctcagtacaatctgctctgatgccgcatagttaagccagccccgacacccgccaacacccgctgacgcgccctgacgggcttgtctgctcccggcatccgcttacagacaagctgtgaccgtctccgggagctgcatgtgtcagaggttttcaccgtcatcaccgaaacgcgcgagacgaaagggcctcgtgatacgcctatttttataggttaatgtcatgataataatggtttcttagacgtcaggtggcacttttcggggaaatgtgcgcggaacccctatttgtttatttttctaaatacattcaaatatgtatccgctcatgagacaataaccctgataaatgcttcaataatattgaaaaaggaagagtatgagtattcaacatttccgtgtcgcccttattcccttttttgcggcattttgccttcctgtttttgctcacccagaaacgctggtgaaagtaaaagatgctgaagatcagttgggtgcacgagtgggttacatcgaactggatctcaacagcggtaagatccttgagagttttcgccccgaagaacgttttccaatgatgagcacttttaaagttctgctatgtggcgcggtattatcccgtattgacgccgggcaagagcaactcggtcgccgcatacactattctcagaatgacttggttgagtactcaccagtcacagaaaagcatcttacggatggcatgacagtaagagaattatgcagtgctgccataaccatgagtgataacactgcggccaacttacttctgacaacgatcggaggaccgaaggagctaaccgcttttttgcacaacatgggggatcatgtaactcgccttgatcgttgggaaccggagctgaatgaagccataccaaacgacgagcgtgacaccacgatgcctgtagcaatggcaacaacgttgcgcaaactattaactggcgaactacttactctagcttcccggcaacaattaatagactggatggaggcggataaagttgcaggaccacttctgcgctcggcccttccggctggctggtttattgctgataaatctggagccggtgagcgtgggtctcgcggtatcattgcagcactggggccagatggtaagccctcccgtatcgtagttatctacacgacggggagtcaggcaactatggatgaacgaaatagacagatcgctgagataggtgcctcactgattaagcattggtaactgtcagaccaagtttactcatatatactttagattgatttaaaacttcatttttaatttaaaaggatctaggtgaagatcctttttgataatctcatgaccaaaatcccttaacgtgagttttcgttccactgagcgtcagaccccgtagaaaagatcaaaggatcttcttgagatcctttttttctgcgcgtaatctgctgcttgcaaacaaaaaaaccaccgctaccagcggtggtttgtttgccggatcaagagctaccaactctttttccgaaggtaactggcttcagcagagcgcagataccaaatactgttcttctagtgtagccgtagttaggccaccacttcaagaactctgtagcaccgcctacatacctcgctctgctaatcctgttaccagtggctgctgccagtggcgataagtcgtgtcttaccgggttggactcaagacgatagttaccggataaggcgcagcggtcgggctgaacggggggttcgtgcacacagcccagcttggagcgaacgacctacaccgaactgagatacctacagcgtgagctatgagaaagcgccacgcttcccgaagggagaaaggcggacaggtatccggtaagcggcagggtcggaacaggagagcgcacgagggagcttccagggggaaacgcctggtatctttatagtcctgtcgggtttcgccacctctgacttgagcgtcgatttttgtgatgctcgtcaggggggcggagcctatggaaaaacgccagcaacgcggcctttttacggttcctggccttttgctggccttttgctcacatgttctttcctgcgttatcccctgattctgtggataaccgtattaccgcctttgagtgagctgataccgctcgccgcagccgaacgaccgagcgcagcgagtcagtgagcgaggaagcggaagagcgcccaatacgcaaaccgcctctccccgcgcgttggccgattcattaatgcagctggcacgacaggtttcccgactggaaagcgggcagtgagcgcaacgcaattaatgtgagttagctcactcattaggcaccccaggctttacactttatgcttccggctcgtatgttgtgtggaattgtgagcggataacaatttcacacaggaaacagctatgaccatgattacgaatt

SEQ ID NO: 51 - DNA, 4242 bp, Artificial Sequence
  pGL4.10 backbone vector
ggcctaactggccggtacctgagctcgctagcctcgaggatatcaagatctggcctcggcggccaagcttggcaatccggtactgttggtaaagccaccatggaagatgccaaaaacattaagaagggcccagcgccattctacccactcgaagacgggaccgccggcgagcagctgcacaaagccatgaagcgctacgccctggtgcccggcaccatcgcctttaccgacgcacatatcgaggtggacattacctacgccgagtacttcgagatgagcgttcggctggcagaagctatgaagcgctatgggctgaatacaaaccatcggatcgtggtgtgcagcgagaatagcttgcagttcttcatgcccgtgttgggtgccctgttcatcggtgtggctgtggccccagctaacgacatctacaacgagcgcgagctgctgaacagcatgggcatcagccagcccaccgtcgtattcgtgagcaagaaagggctgcaaaagatcctcaacgtgcaaaagaagctaccgatcatacaaaagatcatcatcatggatagcaagaccgactaccagggcttccaaagcatgtacaccttcgtgacttcccatttgccacccggcttcaacgagtacgacttcgtgcccgagagcttcgaccgggacaaaaccatcgccctgatcatgaacagtagtggcagtaccggattgcccaagggcgtagccctaccgcaccgcaccgcttgtgtccgattcagtcatgcccgcgaccccatcttcggcaaccagatcatccccgacaccgctatcctcagcgtggtgccatttcaccacggcttcggcatgttcaccacgctgggctacttgatctgcggctttcgggtcgtgctcatgtaccgcttcgaggaggagctattcttgcgcagcttgcaagactataagattcaatctgccctgctggtgcccacactatttagcttcttcgctaagagcactctcatcgacaagtacgacctaagcaacttgcacgagatcgccagcggcggggcgccgctcagcaaggaggtaggtgaggccgtggccaaacgcttccacctaccaggcatccgccagggctacggcctgacagaaacaaccagcgccattctgatcacccccgaaggggacgacaagcctggcgcagtaggcaaggtggtgcccttcttcgaggctaaggtggtggacttggacaccggtaagacactgggtgtgaaccagcgcggcgagctgtgcgtccgtggccccatgatcatgagcggctacgttaacaaccccgaggctacaaacgctctcatcgacaaggacggctggctgcacagcggcgacatcgcctactgggacgaggacgagcacttcttcatcgtggaccggctgaagagcctgatcaaatacaagggctaccaggtagccccagccgaactggagagcatcctgctgcaacaccccaacatcttcgacgccggggtcgccggcctgcccgacgacgatgccggcgagctgcccgccgcagtcgtcgtgctggaacacggtaaaaccatgaccgagaaggagatcgtggactatgtggccagccaggttacaaccgccaagaagctgcgcggtggtgttgtgttcgtggacgaggtgcctaaaggactgaccggcaagttggacgcccgcaagatccgcgagattctcattaaggccaagaagggcggcaagatcgccgtgtaataattctagagtcggggcggccggccgcttcgagcagacatgataagatacattgatgagtttggacaaaccacaactagaatgcagtgaaaaaaatgctttatttgtgaaatttgtgatgctattgctttatttgtaaccattataagctgcaataaacaagttaacaacaacaattgcattcattttatgtttcaggttcagggggaggtgtgggaggttttttaaagcaagtaaaacctctacaaatgtggtaaaatcgataaggatccgtcgaccgatgcccttgagagccttcaacccagtcagctccttccggtgggcgcggggcatgactatcgtcgccgcacttatgactgtcttctttatcatgcaactcgtaggacaggtgccggcagcgctcttccgcttcctcgctcactgactcgctgcgctcggtcgttcggctgcggcgagcggtatcagctcactcaaaggcggtaatacggttatccacagaatcaggggataacgcaggaaagaacatgtgagcaaaaggccagcaaaaggccaggaaccgtaaaaaggccgcgttgctggcgtttttccataggctccgcccccctgacgagcatcacaaaaatcgacgctcaagtcagaggtggcgaaacccgacaggactataaagataccaggcgtttccccctggaagctccctcgtgcgctctcctgttccgaccctgccgcttaccggatacctgtccgcctttctcccttcgggaagcgtggcgctttctcatagctcacgctgtaggtatctcagttcggtgtaggtcgttcgctccaagctgggctgtgtgcacgaaccccccgttcagcccgaccgctgcgccttatccggtaactatcgtcttgagtccaacccggtaagacacgacttatcgccactggcagcagccactggtaacaggattagcagagcgaggtatgtaggcggtgctacagagttcttgaagtggtggcctaactacggctacactagaagaacagtatttggtatctgcgctctgctgaagccagttaccttcggaaaaagagttggtagctcttgatccggcaaacaaaccaccgctggtagcggtggtttttttgtttgcaagcagcagattacgcgcagaaaaaaaggatctcaagaagatcctttgatcttttctacggggtctgacgctcagtggaacgaaaactcacgttaagggattttggtcatgagattatcaaaaaggatcttcacctagatccttttaaattaaaaatgaagttttaaatcaatctaaagtatatatgagtaaacttggtctgacagcggccgcaaatgctaaaccactgcagtggttaccagtgcttgatcagtgaggcaccgatctcagcgatctgcctatttcgttcgtccatagtggcctgactccccgtcgtgtagatcactacgattcgtgagggcttaccatcaggccccagcgcagcaatgatgccgcgagagccgcgttcaccggcccccgatttgtcagcaatgaaccagccagcagggagggccgagcgaagaagtggtcctgctactttgtccgcctccatccagtctatgagctgctgtcgtgatgctagagtaagaagttcgccagtgagtagtttccgaagagttgtggccattgctactggcatcgtggtatcacgctcgtcgttcggtatggcttcgttcaactctggttcccagcggtcaagccgggtcacatgatcacccatattatgaagaaatgcagtcagctccttagggcctccgatcgttgtcagaagtaagttggccgcggtgttgtcgctcatggtaatggcagcactacacaattctcttaccgtcatgccatccgtaagatgcttttccgtgaccggcgagtactcaaccaagtcgttttgtgagtagtgtatacggcgaccaagctgctcttgcccggcgtctatacgggacaacaccgcgccacatagcagtactttgaaagtgctcatcatcgggaatcgttcttcggggcggaaagactcaaggatcttgccgctattgagatccagttcgatatagcccactcttgcacccagttgatcttcagcatcttttactttcaccagcgtttcggggtgtgcaaaaacaggcaagcaaaatgccgcaaagaagggaatgagtgcgacacgaaaatgttggatgctcatactcgtcctttttcaatattattgaagcatttatcagggttactagtacgtctctcaaggataagtaagtaatattaaggtacgggaggtattggacaggccgcaataaaatatctttattttcattacatctgtgtgttggttttttgtgtgaatcgatagtactaacatacgctctccatcaaaacaaaacgaaacaaaacaaactagcaaaataggctgtccccagtgcaagtgcaggtgccagaacatttctct

SEQ ID NO: 52 - DNA, 584 bp, Artificial Sequence
  CMV-IE comparative promoter
gacattgattattgactagttattaatagtaatcaattacggggtcattagttcatagcccatatatggagttccgcgttacataacttacggtaaatggcccgcctggctgaccgcccaacgacccccgcccattgacgtcaataatgacgtatgttcccatagtaacgccaatagggactttccattgacgtcaatgggtggagtatttacggtaaactgcccacttggcagtacatcaagtgtatcatatgccaagtacgccccctattgacgtcaatgacggtaaatggcccgcctggcattatgcccagtacatgaccttatgggactttcctacttggcagtacatctacgtattagtcatcgctattaccatggtgatgcggttttggcagtacatcaatgggcgtggatagcggtttgactcacggggatttccaagtctccaccccattgacgtcaatgggagtttgttttggcaccaaaatcaacgggactttccaaaatgtcgtaacaactccgccccattgacgcaaatgggcggtaggcgtgtacggtgggaggtctatataagcagagct

SEQ ID NO: 53 - DNA, 8191 bp, Artificial Sequence
  pcDNA6.0 beta-galactosidase transfection control
gacggatcgggagatctcccgatcccctatggtgcactctcagtacaatctgctctgatgccgcatagttaagccagtatctgctccctgcttgtgtgttggaggtcgctgagtagtgcgcgagcaaaatttaagctacaacaaggcaaggcttgaccgacaattgcatgaagaatctgcttagggttaggcgttttgcgctgcttcgcgatgtacgggccagatatacgcgttgacattgattattgactagttattaatagtaatcaattacggggtcattagttcatagcccatatatggagttccgcgttacataacttacggtaaatggcccgcctggctgaccgcccaacgacccccgcccattgacgtcaataatgacgtatgttcccatagtaacgccaatagggactttccattgacgtcaatgggtggagtatttacggtaaactgcccacttggcagtacatcaagtgtatcatatgccaagtacgccccctattgacgtcaatgacggtaaatggcccgcctggcattatgcccagtacatgaccttatgggactttcctacttggcagtacatctacgtattagtcatcgctattaccatggtgatgcggttttggcagtacatcaatgggcgtggatagcggtttgactcacggggatttccaagtctccaccccattgacgtcaatgggagtttgttttggcaccaaaatcaacgggactttccaaaatgtcgtaacaactccgccccattgacgcaaatgggcggtaggcgtgtacggtgggaggtctatataagcagagctctctggctaactagagaacccactgcttactggcttatcgaaattaatacgactcactatagggagacccaagctggctagcgtttaaacttaagcttggtaccgagctcggatccactagtccagtgtggtggaattctgcagatcgaaacgatgatagatcccgtcgttttacaacgtcgtgactgggaaaaccctggcgttacccaacttaatcgccttgcagcacatccccctttcgccagctggcgtaatagcgaagaggcccgcaccgatcgcccttcccaacagttgcgcagcctgaatggcgaatggcgctttgcctggtttccggcaccagaagcggtgccggaaagctggctggagtgcgatcttcctgaggccgatactgtcgtcgtcccctcaaactggcagatgcacggttacgatgcgcccatctacaccaacgtgacctatcccattacggtcaatccgccgtttgttcccacggagaatccgacgggttgttactcgctcacatttaatgttgatgaaagctggctacaggaaggccagacgcgaattatttttgatggcgttaactcggcgtttcatctgtggtgcaacgggcgctgggtcggttacggccaggacagtcgtttgccgtctgaatttgacctgagcgcatttttacgcgccggagaaaaccgcctcgcggtgatggtgctgcgctggagtgacggcagttatctggaagatcaggatatgtggcggatgagcggcattttccgtgacgtctcgttgctgcataaaccgactacacaaatcagcgatttccatgttgccactcgctttaatgatgatttcagccgcgctgtactggaggctgaagttcagatgtgcggcgagttgcgtgactacctacgggtaacagtttctttatggcagggtgaaacgcaggtcgccagcggcaccgcgcctttcggcggtgaaattatcgatgagcgtggtggttatgccgatcgcgtcacactacgtctgaacgtcgaaaacccgaaactgtggagcgccgaaatcccgaatctctatcgtgcggtggttgaactgcacaccgccgacggcacgctgattgaagcagaagcctgcgatgtcggtttccgcgaggtgcggattgaaaatggtctgctgctgctgaacggcaagccgttgctgattcgaggcgttaaccgtcacgagcatcatcctctgcatggtcaggtcatggatgagcagacgatggtgcaggatatcctgctgatgaagcagaacaactttaacgccgtgcgctgttcgcattatccgaaccatccgctgtggtacacgctgtgcgaccgctacggcctgtatgtggtggatgaagccaatattgaaacccacggcatggtgccaatgaatcgtctgaccgatgatccgcgctggctaccggcgatgagcgaacgcgtaacgcgaatggtgcagcgcgatcgtaatcacccgagtgtgatcatctggtcgctggggaatgaatcaggccacggcgctaatcacgacgcgctgtatcgctggatcaaatctgtcgatccttcccgcccggtgcagtatgaaggcggcggagccgacaccacggccaccgatattatttgcccgatgtacgcgcgcgtggatgaagaccagcccttcccggctgtgccgaaatggtccatcaaaaaatggctttcgctacctggagagacgcgcccgctgatcctttgcgaatacgcccacgcgatgggtaacagtcttggcggtttcgctaaatactggcaggcgtttcgtcagtatccccgtttacagggcggcttcgtctgggactgggtggatcagtcgctgattaaatatgatgaaaacggcaacccgtggtcggcttacggcggtgattttggcgatacgccgaacgatcgccagttctgtatgaacggtctggtctttgccgaccgcacgccgcatccagcgctgacggaagcaaaacaccagcagcagtttttccagttccgtttatccgggcaaaccatcgaagtgaccagcgaatacctgttccgtcatagcgataacgagctcctgcactggatggtggcgctggatggtaagccgctggcaagcggtgaagtgcctctggatgtcgctccacaaggtaaacagttgattgaactgcctgaactaccgcagccggagagcgccgggcaactctggctcacagtacgcgtagtgcaaccgaacgcgaccgcatggtcagaagccgggcacatcagcgcctggcagcagtggcgtctggcggaaaacctcagtgtgacgctccccgccgcgtcccacgccatcccgcatctgaccaccagcgaaatggatttttgcatcgagctgggtaataagcgttggcaatttaaccgccagtcaggctctctttcacagatgtggattggcgataaaaaccaactgctgacgccgctgcgcgatcagttcacccgtgcaccgctggataacgacattggcgtaagtgaagcgacccgcattgaccctaacgcctgggtcgaacgctggaaggcggcgggccattaccaggccgaagcagcgttgttgcagtgcacggcagatacacttgctgatgcggtgctgattacgaccgctcacgcgtggcagcatcaggggaaaaccttatttatcagccggaaaacctaccggattgatggtagtggtcaaatggcgattaccgttgatgttgaagtggcgagcgatacaccgcatccggcgcggattggcctgaactgccagctggcgcaggtagcagagcgggtaaactggctcggattagggccgcaagaaaactatcccgaccgccttactgccgcctgttttgaccgctgggatctgccattgtcagacatgtataccccgtacgtcttcccgagcgaaaacggtctgcgctgcgggacgcgcgaattgaattatggcccacaccagtggcgcggcgacttccagttcaacatcagccgctacagtcaacagcaactgatggaaaccagccatcgccatctgctgcacgcggaagaaggcacatggctgaatatcgacggtttccatatggggattggtggcgacgactcctggagcccgtcagtatcggcggaattccagctgagcgccggtcgctaccattaccagttggtctggtgtcaaaaagcggccgctcgaggtcacccattcgaaggtaagcctatccctaaccctctcctcggtctcgattctacgcgtaccggtcatcatcaccatcaccattgagtttaaacccgctgatcagcctcgactgtgccttctagttgccagccatctgttgtttgcccctcccccgtgccttccttgaccctggaaggtgccactcccactgtcctttcctaataaaatgaggaaattgcatcgcattgtctgagtaggtgtcattctattctggggggtggggtggggcaggacagcaagggggaggattgggaagacaatagcaggcatgctggggatgcggtgggctctatggcttctgaggcggaaagaaccagctggggctctagggggtatccccacgcgccctgtagcggcgcattaagcgcggcgggtgtggtggttacgcgcagcgtgaccgctacacttgccagcgccctagcgcccgctcctttcgctttcttcccttcctttctcgccacgttcgccggctttccccgtcaagctctaaatcgggggctccctttagggttccgatttagtgctttacggcacctcgaccccaaaaaacttgattagggtgatggttcacgtagtgggccatcgccctgatagacggtttttcgccctttgacgttggagtccacgttctttaatagtggactcttgttccaaactggaacaacactcaaccctatctcggtctattcttttgatttataagggattttgccgatttcggcctattggttaaaaaatgagctgatttaacaaaaatttaacgcgaattaattctgtggaatgtgtgtcagttagggtgtggaaagtccccaggctccccagcaggcagaagtatgcaaagcatgcatctcaattagtcagcaaccaggtgtggaaagtccccaggctccccagcaggcagaagtatgcaaagcatgcatctcaattagtcagcaaccatagtcccgcccctaactccgcccatcccgcccctaactccgcccagttccgcccattctccgccccatggctgactaattttttttatttatgcagaggccgaggccgcctctgcctctgagctattccagaagtagtgaggaggcttttttggaggcctaggcttttgcaaaaagctcccgggagcttgtatatccattttcggatctgatcagcacgtgttgacaattaatcatcggcatagtatatcggcatagtataatacgacaaggtgaggaactaaaccatggccaagcctttgtctcaagaagaatccaccctcattgaaagagcaacggctacaatcaacagcatccccatctctgaagactacagcgtcgccagcgcagctctctctagcgacggccgcatcttcactggtgtcaatgtatatcattttactgggggaccttgtgcagaactcgtggtgctgggcactgctgctgctgcggcagctggcaacctgacttgtatcgtcgcgatcggaaatgagaacaggggcatcttgagcccctgcggacggtgccgacaggtgcttctcgatctgcatcctgggatcaaagccatagtgaaggacagtgatggacagccgacggcagttgggattcgtgaattgctgccctctggttatgtgtgggagggctaagcacttcgtggccgaggagcaggactgacacgtgctacgagatttcgattccaccgccgccttctatgaaaggttgggcttcggaatcgttttccgggacgccggctggatgatcctccagcgcggggatctcatgctggagttcttcgcccaccccaacttgtttattgcagcttataatggttacaaataaagcaatagcatcacaaatttcacaaataaagcatttttttcactgcattctagttgtggtttgtccaaactcatcaatgtatcttatcatgtctgtataccgtcgacctctagctagagcttggcgtaatcatggtcatagctgtttcctgtgtgaaattgttatccgctcacaattccacacaacatacgagccggaagcataaagtgtaaagcctggggtgcctaatgagtgagctaactcacattaattgcgttgcgctcactgcccgctttccagtcgggaaacctgtcgtgccagctgcattaatgaatcggccaacgcgcggggagaggcggtttgcgtattgggcgctcttccgcttcctcgctcactgactcgctgcgctcggtcgttcggctgcggcgagcggtatcagctcactcaaaggcggtaatacggttatccacagaatcaggggataacgcaggaaagaacatgtgagcaaaaggccagcaaaaggccaggaaccgtaaaaaggccgcgttgctggcgtttttccataggctccgcccccctgacgagcatcacaaaaatcgacgctcaagtcagaggtggcgaaacccgacaggactataaagataccaggcgtttccccctggaagctccctcgtgcgctctcctgttccgaccctgccgcttaccggatacctgtccgcctttctcccttcgggaagcgtggcgctttctcatagctcacgctgtaggtatctcagttcggtgtaggtcgttcgctccaagctgggctgtgtgcacgaaccccccgttcagcccgaccgctgcgccttatccggtaactatcgtcttgagtccaacccggtaagacacgacttatcgccactggcagcagccactggtaacaggattagcagagcgaggtatgtaggcggtgctacagagttcttgaagtggtggcctaactacggctacactagaagaacagtatttggtatctgcgctctgctgaagccagttaccttcggaaaaagagttggtagctcttgatccggcaaacaaaccaccgctggtagcggtggtttttttgtttgcaagcagcagattacgcgcagaaaaaaaggatctcaagaagatcctttgatcttttctacggggtctgacgctcagtggaacgaaaactcacgttaagggattttggtcatgagattatcaaaaaggatcttcacctagatccttttaaattaaaaatgaagttttaaatcaatctaaagtatatatgagtaaacttggtctgacagttaccaatgcttaatcagtgaggcacctatctcagcgatctgtctatttcgttcatccatagttgcctgactccccgtcgtgtagataactacgatacgggagggcttaccatctggccccagtgctgcaatgataccgcgagacccacgctcaccggctccagatttatcagcaataaaccagccagccggaagggccgagcgcagaagtggtcctgcaactttatccgcctccatccagtctattaattgttgccgggaagctagagtaagtagttcgccagttaatagtttgcgcaacgttgttgccattgctacaggcatcgtggtgtcacgctcgtcgtttggtatggcttcattcagctccggttcccaacgatcaaggcgagttacatgatcccccatgttgtgcaaaaaagcggttagctccttcggtcctccgatcgttgtcagaagtaagttggccgcagtgttatcactcatggttatggcagcactgcataattctcttactgtcatgccatccgtaagatgcttttctgtgactggtgagtactcaaccaagtcattctgagaatagtgtatgcggcgaccgagttgctcttgcccggcgtcaatacgggataataccgcgccacatagcagaactttaaaagtgctcatcattggaaaacgttcttcggggcgaaaactctcaaggatcttaccgctgttgagatccagttcgatgtaacccactcgtgcacccaactgatcttcagcatcttttactttcaccagcgtttctgggtgagcaaaaacaggaaggcaaaatgccgcaaaaaagggaataagggcgacacggaaatgttgaatactcatactcttcctttttcaatattattgaagcatttatcagggttattgtctcatgagcggatacatatttgaatgtatttagaaaaataaacaaataggggttccgcgcacatttccccgaaaagtgccacctgacgtc

SEQ ID NO: 54 - DNA, 3196 bp, Artificial Sequence
  pGL4.10-CMV-MP-EPO
ggcctaactggccggtaccgtcgacgatatcggatccaggtctatataagcagagctcgtttagtgaaccgtcagatcgcctagatacgccatccacgctgttttgacctccatagaagatcgccaccatgggggtgcacgaatgtcctgcctggctgtggcttctcctgtccctgctgtcgctccctctgggcctcccagtcctgggcgccccaccacgcctcatctgtgacagccgagtcctggagaggtacctcttggaggccaaggaggccgagaatatcacgacgggctgtgctgaacactgcagcttgaatgagaatatcactgtcccagacaccaaagttaatttctatgcctggaagaggatggaggtcgggcagcaggccgtagaagtctggcagggcctggccctgctgtcggaagctgtcctgcggggccaggccctgttggtcaactcttcccagccgtgggagcccctgcagctgcatgtggataaagccgtcagtggccttcgcagcctcaccactctgcttcgggctctgggagcccagaaggaagccatctcccctccagatgcggcctcagctgctccactccgaacaatcactgctgacactttccgcaaactcttccgagtctactccaatttcctccggggaaagctgaagctgtacacaggggaggcctgcaggacaggggacagatgatctagagtcggggcggccggccgcttcgagcagacatgataagatacattgatgagtttggacaaaccacaactagaatgcagtgaaaaaaatgctttatttgtgaaatttgtgatgctattgctttatttgtaaccattataagctgcaataaacaagttaacaacaacaattgcattcattttatgtttcaggttcagggggaggtgtgggaggttttttaaagcaagtaaaacctctacaaatgtggtaaaatcgataaggatccgtcgaccgatgcccttgagagccttcaacccagtcagctccttccggtgggcgcggggcatgactatcgtcgccgcacttatgactgtcttctttatcatgcaactcgtaggacaggtgccggcagcgctcttccgcttcctcgctcactgactcgctgcgctcggtcgttcggctgcggcgagcggtatcagctcactcaaaggcggtaatacggttatccacagaatcaggggataacgcaggaaagaacatgtgagcaaaaggccagcaaaaggccaggaaccgtaaaaaggccgcgttgctggcgtttttccataggctccgcccccctgacgagcatcacaaaaatcgacgctcaagtcagaggtggcgaaacccgacaggactataaagataccaggcgtttccccctggaagctccctcgtgcgctctcctgttccgaccctgccgcttaccggatacctgtccgcctttctcccttcgggaagcgtggcgctttctcatagctcacgctgtaggtatctcagttcggtgtaggtcgttcgctccaagctgggctgtgtgcacgaaccccccgttcagcccgaccgctgcgccttatccggtaactatcgtcttgagtccaacccggtaagacacgacttatcgccactggcagcagccactggtaacaggattagcagagcgaggtatgtaggcggtgctacagagttcttgaagtggtggcctaactacggctacactagaagaacagtatttggtatctgcgctctgctgaagccagttaccttcggaaaaagagttggtagctcttgatccggcaaacaaaccaccgctggtagcggtggtttttttgtttgcaagcagcagattacgcgcagaaaaaaaggatctcaagaagatcctttgatcttttctacggggtctgacgctcagtggaacgaaaactcacgttaagggattttggtcatgagattatcaaaaaggatcttcacctagatccttttaaattaaaaatgaagttttaaatcaatctaaagtatatatgagtaaacttggtctgacagcggccgcaaatgctaaaccactgcagtggttaccagtgcttgatcagtgaggcaccgatctcagcgatctgcctatttcgttcgtccatagtggcctgactccccgtcgtgtagatcactacgattcgtgagggcttaccatcaggccccagcgcagcaatgatgccgcgagagccgcgttcaccggcccccgatttgtcagcaatgaaccagccagcagggagggccgagcgaagaagtggtcctgctactttgtccgcctccatccagtctatgagctgctgtcgtgatgctagagtaagaagttcgccagtgagtagtttccgaagagttgtggccattgctactggcatcgtggtatcacgctcgtcgttcggtatggcttcgttcaactctggttcccagcggtcaagccgggtcacatgatcacccatattatgaagaaatgcagtcagctccttagggcctccgatcgttgtcagaagtaagttggccgcggtgttgtcgctcatggtaatggcagcactacacaattctcttaccgtcatgccatccgtaagatgcttttccgtgaccggcgagtactcaaccaagtcgttttgtgagtagtgtatacggcgaccaagctgctcttgcccggcgtctatacgggacaacaccgcgccacatagcagtactttgaaagtgctcatcatcgggaatcgttcttcggggcggaaagactcaaggatcttgccgctattgagatccagttcgatatagcccactcttgcacccagttgatcttcagcatcttttactttcaccagcgtttcggggtgtgcaaaaacaggcaagcaaaatgccgcaaagaagggaatgagtgcgacacgaaaatgttggatgctcatactcgtcctttttcaatattattgaagcatttatcagggttactagtacgtctctcaaggataagtaagtaatattaaggtacgggaggtattggacaggccgcaataaaatatctttattttcattacatctgtgtgttggttttttgtgtgaatcgatagtactaacatacgctctccatcaaaacaaaacgaaacaaaacaaactagcaaaataggctgtccccagtgcaagtgcaggtgccagaacatttctct

SEQ ID NO: 55 - DNA, 13 bp, Mus musculus
tggcacagtgcca

SEQ ID NO: 56 - DNA, 13 bp, Homo sapiens
tgaagaggtggca

SEQ ID NO: 57 - DNA, 16 bp, Mus musculus
tcaacttgcctgacac

SEQ ID NO: 58 - DNA, 16 bp, Homo sapiens
tggactttcctgaacc

SEQ ID NO: 59 - DNA, 273 bp, Artificial Sequence
  Human NR1x3-Min TK
actgtactttcctgaccctgaagagactgtactttcctgaccctgaagagactgtactttcctgaccctgaagaggatccggccccgcccagcgtcttgtcattggcgaattcgaacacgcagatgcagtcggggcggcgcggtccgaggtccacttcgcatattaaggtgacgcgtgtggcctcgaacaccgagcgaccctgcagcgacccgcttaacagcgtcaacagcgtgccgcagatctcgaggagcttggcgagattttcaggagct

SEQ ID NO: 60 - DNA, 286 bp, Artificial Sequence
  Human PBREM-MinTK
actgtactttcctgaccctgaagaggtggcagcatggactttcctgaaccagatccggccccgcccagcgtcttgtcattggcgaattcgaacacgcagatgcagtcggggcggcgcggtccgaggtccacttcgcatattaaggtgacgcgtgtggcctcgaacaccgagcgaccctgcagcgacccgcttaacagcgtcaacagcgtgccgcagatctcgaggagcttggcgagattttcaggagctaaggaagctaaacatggaagatgccaaaaacattaag

SEQ ID NO: 61 - DNA, 286 bp, Artificial Sequence
  hNR1-mNFI-hNR2-Min TK (HMH MinTK)
actgtactttcctgaccctggcacagtgccaccatggactttcctgaaccagatccggccccgcccagcgtcttgtcattggcgaattcgaacacgcagatgcagtcggggcggcgcggtccgaggtccacttcgcatattaaggtgacgcgtgtggcctcgaacaccgagcgaccctgcagcgacccgcttaacagcgtcaacagcgtgccgcagatctcgaggagcttggcgagattttcaggagctaaggaagctaaacatggaagatgccaaaaacattaag

SEQ ID NO: 62 - DNA, 286 bp, Artificial Sequence
  hNR1-mNFI mNR2-Min TK (HMM MinTK)
actgtactttcctgaccctggcacagtgccaccatcaacttgcctgacaccgatccggccccgcccagcgtcttgtcattggcgaattcgaacacgcagatgcagtcggggcggcgcggtccgaggtccacttcgcatattaaggtgacgcgtgtggcctcgaacaccgagcgaccctgcagcgacccgcttaacagcgtcaacagcgtgccgcagatctcgaggagcttggcgagattttcaggagctaaggaagctaaacatggaagatgccaaaaacattaag

SEQ ID NO: 63 - DNA, 286 bp, Artificial Sequence
  mNR1-hNFI-mNR2-Min TK (MHM MinTK)
tctgtactttcctgaccttgaagaggtggcaccatcaacttgcctgacaccgatccggccccgcccagcgtcttgtcattggcgaattcgaacacgcagatgcagtcggggcggcgcggtccgaggtccacttcgcatattaaggtgacgcgtgtggcctcgaacaccgagcgaccctgcagcgacccgcttaacagcgtcaacagcgtgccgcagatctcgaggagcttggcgagattttcaggagctaaggaagctaaacatggaagatgccaaaaacattaag

SEQ ID NO: 64 - DNA, 286 bp, Artificial Sequence
  mNR1-hNFI hNR2-Min TK (MHH MinTK)
tctgtactttcctgaccttgaagaggtggcagcatggactttcctgaaccagatccggccccgcccagcgtcttgtcattggcgaattcgaacacgcagatgcagtcggggcggcgcggtccgaggtccacttcgcatattaaggtgacgcgtgtggcctcgaacaccgagcgaccctgcagcgacccgcttaacagcgtcaacagcgtgccgcagatctcgaggagcttggcgagattttcaggagctaaggaagctaaacatggaagatgccaaaaacattaag

SEQ ID NO: 65 - DNA, 330 bp, Artificial Sequence
  hPB-SV40
actgtactttcctgaccctgaagaggtggcagcatggactttcctgaaccagctgggagttcgtagacggactagcccgggctcgagatctgcgatctgcatctcaattagtcagcaaccatagtcccgcccctaactccgcccatcccgcccctaactccgcccagttccgcccattctccgccccatcgctgactaattttttttatttatgcagaggccgaggccgcctcggcctctgagctattccagaagtagtgaggaggcttttttggaggcctaggcttttgcaaaaagcttggcattccggtactgttggtaaagccaccc

SEQ ID NO: 66 - DNA, 330 bp, Artificial Sequence
  MHM-SV40
tctgtactttcctgaccttgaagaggtggcaccatcaacttgcctgacaccgctgggagttcgtagacggactagcccgggctcgagatctgcgatctgcatctcaattagtcagcaaccatagtcccgcccctaactccgcccatcccgcccctaactccgcccagttccgcccattctccgccccatcgctgactaattttttttatttatgcagaggccgaggccgcctcggcctctgagctattccagaagtagtgaggaggcttttttggaggcctaggcttttgcaaaaagcttggcattccggtactgttggtaaagccaccc

SEQ ID NO: 67 - DNA, 401 bp, Artificial Sequence
  2xhPB SV40
actgtactttcctgaccctgaagaggtggcagcatggactttcctgaaccacattactcgcatccattctcactgtactttcctgaccctgaagaggtggcagcatggactttcctgaaccagctgggagttcgtagacggactagcccgggctcgagatctgcgatctgcatctcaattagtcagcaaccatagtcccgcccctaactccgcccatcccgcccctaactccgcccagttccgcccattctccgccccatcgctgactaattttttttatttatgcagaggccgaggccgcctcggcctctgagctattccagaagtagtgaggaggcttttttggaggcctaggcttttgcaaaaagcttggcattccggtactgttggtaaagccaccc

SEQ ID NO: 68 - DNA, 353 bp, Artificial Sequence
  2xMHM-MinTK
tctgtactttcctgaccttgaagaggtggcaccatcaacttgcctgacacccattactcgcatccattctctctgtactttcctgaccttgaagaggtggcaccatcaacttgcctgacaccgctgggagttcgtagacggagatccggccccgcccagcgtcttgtcattggcgaattcgaacacgcagatgcagtcggggcggcgcggtccgaggtccacttcgcatattaaggtgacgcgtgtggcctcgaacaccgagcgaccctgcagcgacccgcttaacagcgtcaacagcgtgccgcagatctcgaggagcttggcgagattttcaggagctaaggaagctaaac

SEQ ID NO: 69 - DNA, 401 bp, Artificial Sequence
  2xMHM-SV40
tctgtactttcctgaccttgaagaggtggcaccatcaacttgcctgacacccattactcgcatccattctctctgtactttcctgaccttgaagaggtggcaccatcaacttgcctgacaccgctgggagttcgtagacggactagcccgggctcgagatctgcgatctgcatctcaattagtcagcaaccatagtcccgcccctaactccgcccatcccgcccctaactccgcccagttccgcccattctccgccccatcgctgactaattttttttatttatgcagaggccgaggccgcctcggcctctgagctattccagaagtagtgaggaggcttttttggaggcctaggcttttgcaaaaagcttggcattccggtactgttggtaaagccaccc

SEQ ID NO: 70 - DNA, 424 bp, Artificial Sequence
  3xhPB-minTK
actgtactttcctgaccctgaagaggtggcagcatggactttcctgaaccacattactcgcatccattctcactgtactttcctgaccctgaagaggtggcagcatggactttcctgaaccagcactgaaggtcctcaatcgactgtactttcctgaccctgaagaggtggcagcatggactttcctgaaccagctgggagttcgtagacggagatccggccccgcccagcgtcttgtcattggcgaattcgaacacgcagatgcagtcggggcggcgcggtccgaggtccacttcgcatattaaggtgacgcgtgtggcctcgaacaccgagcgaccctgcagcgacccgcttaacagcgtcaacagcgtgccgcagatctcgaggagcttggcgagattttcaggagctaaggaagctaaac

SEQ ID NO: 71 - DNA, 472 bp, Artificial Sequence
  3xhPB-SV40
actgtactttcctgaccctgaagaggtggcagcatggactttcctgaaccacattactcgcatccattctcactgtactttcctgaccctgaagaggtggcagcatggactttcctgaaccagcactgaaggtcctcaatcgactgtactttcctgaccctgaagaggtggcagcatggactttcctgaaccagctgggagttcgtagacggactagcccgggctcgagatctgcgatctgcatctcaattagtcagcaaccatagtcccgcccctaactccgcccatcccgcccctaactccgcccagttccgcccattctccgccccatcgctgactaattttttttatttatgcagaggccgaggccgcctcggcctctgagctattccagaagtagtgaggaggcttttttggaggcctaggcttttgcaaaaagcttggcattccggtactgttggtaaagccaccc

SEQ ID NO: 72 - DNA, 51 bp, Artificial Sequence
  HMH hybrid
actgtactttcctgaccctggcacagtgccaccatggactttcctgaacca

SEQ ID NO: 73 - DNA, 51 bp, Artificial Sequence
  HMM hybrid
actgtactttcctgaccctggcacagtgccaccatcaacttgcctgacacc

SEQ ID NO: 74 - DNA, 51 bp, Artificial Sequence
  MHM hybrid
tctgtactttcctgaccttgaagaggtggcaccatcaacttgcctgacacc

SEQ ID NO: 75 - DNA, 51 bp, Artificial Sequence
  MHH hybrid
tctgtactttcctgaccttgaagaggtggcagcatggactttcctgaacca

SEQ ID NO: 76 - DNA, 101 bp, Artificial Sequence
  2x mouse PBREM CREs
  misc_feature (51)..(52): optional spacer
tctgtactttcctgaccttggcacagtgccaccatcaacttgcctgacaccctgtactttcctgaccttggcacagtgccaccatcaacttgcctgacacc

SEQ ID NO: 77 - DNA, 204 bp, Artificial Sequence
  3x mouse PBREM CREs
  misc_feature (51)..(52): optional spacer
  misc_feature (102)..(103): optional spacer
  misc_feature (153)..(154): optional spacer
tctgtactttcctgaccttggcacagtgccaccatcaacttgcctgacacctctgtactttcctgaccttggcacagtgccaccatcaacttgcctgacacctctgtactttcctgaccttggcacagtgccaccatcaacttgcctgacacctctgtactttcctgaccttggcacagtgccaccatcaacttgcctgacacc

SEQ ID NO: 78 - DNA, 101 bp, Artificial Sequence
  2x MHM hybrids CREs
  misc_feature (50)..(51): optional spacer
ctgtactttcctgaccttgaagaggtggcaccatcaacttgcctgacacctctgtactttcctgaccttgaagaggtggcaccatcaacttgcctgacacc

SEQ ID NO: 79 - DNA, 102 bp, Artificial Sequence; identical to SEQ ID NO: 47
  2x human PBREM CREs
  misc_feature (51)..(52): optional spacer

SEQ ID NO: 80 - DNA, 153 bp, Artificial Sequence; identical to SEQ ID NO: 46
  3x human PBREM CREs
  misc_feature (51)..(52): optional spacer
  misc_feature (102)..(103): optional spacer

SEQ ID NO: 81 - DNA, 122 bp, Artificial Sequence
  2x mouse PBREM CREs
tctgtactttcctgaccttggcacagtgccaccatcaacttgcctgacacccattactcgcatccattctctctgtactttcctgaccttggcacagtgccaccatcaacttgcctgacacc

SEQ ID NO: 82 - DNA, 264 bp, Artificial Sequence
  3x mouse PBREM
tctgtactttcctgaccttggcacagtgccaccatcaacttgcctgacacccattactcgcatccattctctctgtactttcctgaccttggcacagtgccaccatcaacttgcctgacaccgcactgaaggtcctcaatcgtctgtactttcctgaccttggcacagtgccaccatcaacttgcctgacaccctgacctcctgccagcaatatctgtactttcctgaccttggcacagtgccaccatcaacttgcctgacacc

SEQ ID NO: 83 - DNA, 121 bp, Artificial Sequence
  2x MHM hybrids
ctgtactttcctgaccttgaagaggtggcaccatcaacttgcctgacacccattactcgcatccattctctctgtactttcctgaccttgaagaggtggcaccatcaacttgcctgacacc

SEQ ID NO: 84 - DNA, 122 bp, Artificial Sequence
  2x human PBREM
actgtactttcctgaccctgaagaggtggcagcatggactttcctgaaccacattactcgcatccattctcactgtactttcctgaccctgaagaggtggcagcatggactttcctgaacca

SEQ ID NO: 85 - DNA, 193 bp, Artificial Sequence
  3x human PBREM
actgtactttcctgaccctgaagaggtggcagcatggactttcctgaaccacattactcgcatccattctcactgtactttcctgaccctgaagaggtggcagcatggactttcctgaaccagcactgaaggtcctcaatcgactgtactttcctgaccctgaagaggtggcagcatggactttcctgaacca

SEQ ID NO: 86 - DNA, 18 bp, Mus musculus
tctgtactttcctgacct

SEQ ID NO: 87 - DNA, 18 bp, Homo sapiens
actgtactttcctgaccc

SEQ ID NO: 88 - DNA, 16 bp, Mus musculus
tggcacagtgccacca

SEQ ID NO: 89 - DNA, 16 bp, Homo sapiens
tgaagaggtggcagca

SEQ ID NO: 90 - DNA, 17 bp, Mus musculus
tcaacttgcctgacacc

SEQ ID NO: 91 - DNA, 17 bp, Homo sapiens
tggactttcctgaacca